European Patent Application EP 4 378 473 A1, published June 5, 2024. Title: HER2 VACCINE COMPOSITION. Applicant: ASTON SCI. INC. The sequence listing filed with the application follows.

SEQUENCE LISTING (3 sequences)

SEQ ID NO: 1 - protein, 1254 aa, Homo sapiens
MELAALCRWGLLLALLPPGAASTQVCTGTDMKLRLPASPETHLDMLRHLYQGCQVVQGNLELTYLPTNASLSFLQDIQEVQGYVLIAHNQVRQVPLQRLRIVRGTQLFEDNYALAVLDNGDPLNNTTPVTGASPGGLRELQLRSLTEILKGGVLIQRNPQLCYQDTILWKDIFHKNNQLALTLIDTNRSRACHPCSPMCKGSRCWGESSEDCQSLTRTVCAGGCARCKGPLPTDCCHEQCAAGCTGPKHSDCLACLHFNHSGICELHCPALVTYNTDTFESMPNPEGRYTFGASVTACPYNYLSTDVGSCTLVCPLHNQEVTAEDGTQRCEKCSKPCARVCYGLGMEHLREVRAVTSANIQEFAGCKKIFGSLAFLPESFDGDPASNTAPLQPEQLQVFETLEEITGYLYISAWPDSLPDLSVFQNLQVIRGRILHNGAYSLTLQGLGISWLGLRSLRELGSGLALIHHNTHLCFVHTVPWDQLFRNPHQALLHTANRPEDECVGEGLACHQLCARGHCWGPGPTQCVNCSQFLRGQECVEECRVLQGLPREYVNARHCLPCHPECQPQNGSVTCFGPEADQCVACAHYKDPPFCVARCPSGVKPDLSYMPIWKFPDEEGACQPCPINCTHSCVDLDDKGCPAEQRASPLTSIISAVVGILLVVVLGVVFGILIKRRQQKIRKYTMRRLLQETELVEPLTPSGAMPNQAQMRILKETELRKVKVLGSGAFGTVYKGIWIPDGENVKIPVAIKVLRENTSPKANKEILDEAYVMAGVGSPYVSRLLGICLTSTVQLVTQLMPYGCLLDHVRENRGRLGSQDLLNWCMQIAKGMSYLEDVRLVHRDLAARNVLVKSPNHVKITDFGLARLLDIDETEYHADGGKVPIKWMALESILRRRFTHQSDVWSYGVTVWELMTFGAKPYDGIPAREIPDLLEKGERLPQPPICTIDVYMIMVKCWMIDSECRPRFRELVSEFSRMARDPQRFVVIQNEDLGPASPLDSTFYRSLLEDDDMGDLVDAEEYLVPQQGFFCPDPAPGAGGMVHHRHRSSSTRSGGGDLTLGLEPSEEEAPRSPLAPSEGAGSDVFDGDLGMGAAKGLQSLPTHDPSPLQRYSEDPTVPLPSETDGYVAPLTCSPQPEYVNQPDVRPQPPSPREGPLPAARPAGATLERPKTLSPGKNGVVKDVFAFGGAVENPEYLTPQGGAAPQPHPPPAFSPAFDNLYYWDQDPPERGAPPSTFKGTPTAENPEYLGLDVPV

SEQ ID NO: 2 - protein, 581 aa, Homo sapiens
MKRRQQKIRKYTMRRLLQETELVEPLTPSGAMPNQAQMRILKETELRKVKVLGSGAFGTVYKGIWIPDGENVKIPVAIKVLRENTSPKANKEILDEAYVMAGVGSPYVSRLLGICLTSTVQLVTQLMPYGCLLDHVRENRGRLGSQDLLNWCMQIAKGMSYLEDVRLVHRDLAARNVLVKSPNHVKITDFGLARLLDIDETEYHADGGKVPIKWMALESILRRRFTHQSDVWSYGVTVWELMTFGAKPYDGIPAREIPDLLEKGERLPQPPICTIDVYMIMVKCWMIDSECRPRFRELVSEFSRMARDPQRFVVIQNEDLGPASPLDSTFYRSLLEDDDMGDLVDAEEYLVPQQGFFCPDPAPGAGGMVHHRHRSSSTRSGGGDLTLGLEPSEEEAPRSPLAPSEGAGSDVFDGDLGMGAAKGLQSLPTHDPSPLQRYSEDPTVPLPSETDGYVAPLTCSPQPEYVNQPDVRPQPPSPREGPLPAARPAGATLERAKTLSPGKNGVVKDVFAFGGAVENPEYLTPQGGAAPQPHPPPAFSPAFDNLYYWDQDPPERGAPPSTFKGTPTAENPEYLGLDVPV

SEQ ID NO: 3 - DNA, 1746 bp, Homo sapiens
  source 1..1746: mol_type = genomic DNA
atgaagcgacggcagcagaagatccggaagtacacgatgcggagactgctgcaggaaacggagctggtggagccgctgacacctagcggagcgatgcccaaccaggcgcagatgcggatcctgaaagagacggagctgaggaaggtgaaggtgcttggatctggcgcttttggcacagtctacaagggcatctggatccctgatggggagaatgtgaaaattccagtggccatcaaagtgttgagggaaaacacatcccccaaagccaacaaagaaatcttagacgaagcatacgtgatggctggtgtgggctccccatatgtctcccgccttctgggcatctgcctgacatccacggtgcagctggtgacacagcttatgccctatggctgcctcttagaccatgtccgggaaaaccgcggacgcctgggctcccaggacctgctgaactggtgtatgcagattgccaaggggatgagctacctggaggatgtgcggctcgtacacagggacttggccgctcggaacgtgctggtcaagagtcccaaccatgtcaaaattacagacttcgggctggctcggctgctggacattgacgagacagagtaccatgcagatgggggcaaggtgcccatcaagtggatggcgctggagtccattctccgccggcggttcacccaccagagtgatgtgtggagttatggtgtgactgtgtgggagctgatgacttttggggccaaaccttacgatgggatcccagcccgggagatccctgacctgctggaaaagggggagcggctgccccagccccccatctgcaccattgatgtctacatgatcatggtcaaatgttggatgattgactctgaatgtcggccaagattccgggagttggtgtctgaattctcccgcatggccagggacccccagcgctttgtggtcatccagaatgaggacttgggcccagccagtcccttggacagcaccttctaccgctcactgctggaggacgatgacatgggggacctggtggatgctgaggagtatctggtaccccagcagggcttcttctgtccagaccctgccccgggcgctgggggcatggtccaccacaggcaccgcagctcatctaccaggagtggcggtggggacctgacactagggctggagccctctgaagaggaggcccccaggtctccactggcaccctccgaaggggctggctccgatgtatttgatggtgacctgggaatgggggcagccaaggggctgcaaagcctccccacacatgaccccagccctctacagcggtacagtgaggaccccacagtacccctgccctctgagactgatggctacgttgcccccctgacctgcagcccccagcctgaatatgtgaaccagccagatgttcggccccagcccccttcgccccgagagggccctctgcctgctgcccgacctgctggtgccactctggaaagggccaagactctctccccagggaagaatggggtcgtcaaagacgtttttgcctttgggggtgccgtggagaaccccgagtacttgacaccccagggaggagctgcccctcagccccaccctcctcctgccttcagcccagccttcgacaacctctattactgggaccaggacccaccagagcggggggctccacccagcaccttcaaagggacacctacggcagagaacccagagtacctgggtctggacgtgccagtgtaa